European Patent Application EP 4 378 486 A1, published June 5, 2024. Title: Secreted splicing variant of Klotho for extending lifespan. Applicant: UNIVERSITAT AUTÒNOMA DE BARCELONA. The sequence listing filed with the application follows.

SEQUENCE LISTING (14 sequences)

SEQ ID NO: 1 - protein, 549 aa, Homo sapiens
MPASAPPRRPRPPPPSLSLLLVLLGLGGRRLRAEPGDGAQTWARVSRPPAPEAAGLFQGTFPDGFLWAVGSAAYQTEGGWQQHGKGASIWDTFTHHPLAPPGDSRNASLPLGAPSPLQPATGDVASDSYNNVFRDTEALRELGVTHYRFSISWARVLPNGSAGVPNREGLRYYRRLLERLRELGVQPVVTLYHWDLPQRLQDAYGGWANRALADHFRDYAELCFRHFGGQVKYWITIDNPYVVAWHGYATGRLAPGIRGSPRLGYLVAHNLLLAHAKVWHLYNTSFRPTQGGQVSIALSSHWINPRRMTDHSIKECQKSLDFVLGWFAKPVFIDGDYPESMKNNLSSILPDFTESEKKFIKGTADFFALCFGPTLSFQLLDPHMKFRQLESPNLRQLLSWIDLEFNHPQIFIVENGWFVSGTTKRDDAKYMYYLKKFIMETLKAIKLDGVDVIGYTAWSLMDGFEWHRGYSIRRGLFYVDFLSQDKMLLPKSSALFYQKLIEKNGFPPLPENQPLEGTFPCDFAWGVVDNYIQVSQLTKPISSLTKPYH

SEQ ID NO: 2 - protein, 550 aa, Mus musculus
MLARAPPRRPPRLVLLRLLLLHLLLLALRARCLSAEPGQGAQTWARFARAPAPEAAGLLHDTFPDGFLWAVGSAAYQTEGGWRQHGKGASIWDTFTHHSGAAPSDSPIVVAPSGAPSPPLSSTGDVASDSYNNVYRDTEGLRELGVTHYRFSISWARVLPNGTAGTPNREGLRYYRRLLERLRELGVQPVVTLYHWDLPQRLQDTYGGWANRALADHFRDYAELCFRHFGGQVKYWITIDNPYVVAWHGYATGRLAPGVRGSSRLGYLVAHNLLLAHAKVWHLYNTSFRPTQGGRVSIALSSHWINPRRMTDYNIRECQKSLDFVLGWFAKPIFIDGDYPESMKNNLSSLLPDFTESEKRLIRGTADFFALSFGPTLSFQLLDPNMKFRQLESPNLRQLLSWIDLEYNHPPIFIVENGWFVSGTTKRDDAKYMYYLKKFIMETLKAIRLDGVDVIGYTAWSLMDGFEWHRGYSIRRGLFYVDFLSQDKELLPKSSALFYQKLIEDNGFPPLPENQPLEGTFPCDFAWGVVDNYVQVSPLTKPSVGLLLPH

SEQ ID NO: 3 - DNA, 1650 bp, Homo sapiens
  source 1..1650: mol_type = other DNA
atgcccgccagcgccccgccgcgccgcccgcgtccaccgccgccgtcgctgtcgctgctgctggtgctgctgggcctgggcggacgacgcctgcgtgcggagccgggcgacggcgcgcagacctgggcccgtgtctcgcggcctcctgcccccgaggccgcgggcctcttccagggcaccttccccgacggcttcctctgggccgtgggcagcgccgcctaccagaccgagggcggctggcagcagcacggcaagggtgcgtccatctgggacacgttcacccaccaccccctggcacccccgggagactcccggaacgccagtctgccgttgggcgccccgtcgccgctgcagcccgccaccggggacgtagccagcgacagctacaacaacgtcttccgcgacacggaggcgctgcgcgagctcggggtcactcactaccgcttctccatctcgtgggcgcgagtgctccccaatggcagcgcgggcgtccccaaccgcgaggggctgcgctactaccggcgcctgctggagcggctgcgggagctgggcgtgcagcccgtggtcaccctgtaccactgggacctgccccagcgcctgcaggacgcctacggcggctgggccaaccgcgccctggccgaccacttcagggattacgcggagctctgcttccgccacttcggcggtcaggtcaagtactggatcaccatcgacaacccctacgtggtggcctggcacggctacgccaccgggcgcctggcccccggcatccggggcagcccgcggctcgggtacctggtggcgcacaacctcctcctggctcatgccaaagtctggcatctctacaatacttctttccgtcccactcagggaggtcaggtgtccattgccctaagctctcactggatcaatcctcgaagaatgaccgaccacagcatcaaagaatgtcaaaaatctctggactttgtactaggttggtttgccaaacccgtatttattgatggtgactatcccgagagcatgaagaataacctttcatctattctgcctgattttactgaatctgagaaaaagttcatcaaaggaactgctgacttttttgctctttgctttggacccaccttgagttttcaacttttggaccctcacatgaagttccgccaattggaatctcccaacctgaggcaactgctttcctggattgaccttgaatttaaccatcctcaaatatttattgtggaaaatggctggtttgtctcagggaccaccaagagagatgatgccaaatatatgtattacctcaaaaagttcatcatggaaaccttaaaagccatcaagctggatggggtggatgtcatcgggtataccgcatggtccctcatggatggtttcgagtggcacagaggttacagcatcaggcgtggactcttctatgttgactttctaagccaggacaagatgttgttgccaaagtcttcagccttgttctaccaaaagctgatagagaaaaatggcttccctcctttacctgaaaatcagcccctagaagggacatttccctgtgactttgcttggggagttgtcgacaactacattcaagtaagtcagctgacaaaaccaatcagcagtctcaccaagccctatcactag

SEQ ID NO: 4 - DNA, 1653 bp, Mus musculus
  source 1..1653: mol_type = other DNA
atgctcgcccgcgcccctcctcgccgcccgccgcggctggtgctgctccgtttgctgttgctgcatctgctgctgctcgccctgcgcgcccgctgcctgagcgctgagccgggtcagggcgcgcagacctgggctcgcttcgcgcgcgctcctgccccagaggccgctggcctcctccacgacaccttccccgacggtttcctctgggcggtaggcagcgccgcctatcagaccgagggcggctggcgacagcacggcaaaggcgcgtccatctgggacactttcacccatcactctggggcggccccgtccgactccccgatcgtcgtggcgccgtcgggtgccccgtcgcctcccctgtcctccactggagatgtggccagcgatagttacaacaacgtctaccgcgacacagaggggctgcgcgaactgggggtcacccactaccgcttctccatatcgtgggcgcgggtgctccccaatggcaccgcgggcactcccaaccgcgaggggctgcgctactaccggcggctgctggagcggctgcgggagctgggcgtgcagccggtggttaccctgtaccattgggacctgccacagcgcctgcaggacacctatggcggatgggccaatcgcgccctggccgaccatttcagggattatgccgagctctgcttccgccacttcggtggtcaggtcaagtactggatcaccattgacaacccctacgtggtggcctggcacgggtatgccaccgggcgcctggccccgggcgtgaggggcagctccaggctcgggtacctggttgcccacaacctacttttggctcatgccaaagtctggcatctctacaacacctctttccgccccacacagggaggccgggtgtctatcgccttaagctcccattggatcaatcctcgaagaatgactgactataatatcagagaatgccagaagtctcttgactttgtgctaggctggtttgccaaacccatatttattgatggcgactacccagagagtatgaagaacaacctctcgtctcttctgcctgattttactgaatctgagaagaggctcatcagaggaactgctgacttttttgctctctccttcggaccaaccttgagctttcagctattggaccctaacatgaagttccgccaattggagtctcccaacctgaggcagcttctgtcttggatagatctggaatataaccaccctccaatatttattgtggaaaatggctggtttgtctcgggaaccaccaaaagggatgatgccaaatatatgtattatctcaagaagttcataatggaaaccttaaaagcaatcagactggatggggtcgacgtcattgggtacaccgcgtggtcgctcatggacggtttcgagtggcataggggctacagcatccggcgaggactcttctacgttgactttctgagtcaggacaaggagctgttgccaaagtcttcggccttgttctaccaaaagctgatagaggacaatggctttcctcctttacctgaaaaccagccccttgaagggacatttccctgtgactttgcttggggagttgttgacaactacgttcagctgagtcctttgacaaaacccagtgtcggcctcttgcttcctcactaa

SEQ ID NO: 5 - protein, 534 aa, Homo sapiens
MPASAPPRRPRPPPPSLSLLLVLLGLGGRRLRAEPGDGAQTWARVSRPPAPEAAGLFQGTFPDGFLWAVGSAAYQTEGGWQQHGKGASIWDTFTHHPLAPPGDSRNASLPLGAPSPLQPATGDVASDSYNNVFRDTEALRELGVTHYRFSISWARVLPNGSAGVPNREGLRYYRRLLERLRELGVQPVVTLYHWDLPQRLQDAYGGWANRALADHFRDYAELCFRHFGGQVKYWITIDNPYVVAWHGYATGRLAPGIRGSPRLGYLVAHNLLLAHAKVWHLYNTSFRPTQGGQVSIALSSHWINPRRMTDHSIKECQKSLDFVLGWFAKPVFIDGDYPESMKNNLSSILPDFTESEKKFIKGTADFFALCFGPTLSFQLLDPHMKFRQLESPNLRQLLSWIDLEFNHPQIFIVENGWFVSGTTKRDDAKYMYYLKKFIMETLKAIKLDGVDVIGYTAWSLMDGFEWHRGYSIRRGLFYVDFLSQDKMLLPKSSALFYQKLIEKNGFPPLPENQPLEGTFPCDFAWGVVDNYIQV

SEQ ID NO: 6 - protein, 536 aa, Mus musculus
MLARAPPRRPPRLVLLRLLLLHLLLLALRARCLSAEPGQGAQTWARFARAPAPEAAGLLHDTFPDGFLWAVGSAAYQTEGGWRQHGKGASIWDTFTHHSGAAPSDSPIVVAPSGAPSPPLSSTGDVASDSYNNVYRDTEGLRELGVTHYRFSISWARVLPNGTAGTPNREGLRYYRRLLERLRELGVQPVVTLYHWDLPQRLQDTYGGWANRALADHFRDYAELCFRHFGGQVKYWITIDNPYVVAWHGYATGRLAPGVRGSSRLGYLVAHNLLLAHAKVWHLYNTSFRPTQGGRVSIALSSHWINPRRMTDYNIRECQKSLDFVLGWFAKPIFIDGDYPESMKNNLSSLLPDFTESEKRLIRGTADFFALSFGPTLSFQLLDPNMKFRQLESPNLRQLLSWIDLEYNHPPIFIVENGWFVSGTTKRDDAKYMYYLKKFIMETLKAIRLDGVDVIGYTAWSLMDGFEWHRGYSIRRGLFYVDFLSQDKELLPKSSALFYQKLIEDNGFPPLPENQPLEGTFPCDFAWGVVDNYVQV

SEQ ID NO: 7 - DNA, 3683 bp, synthetic construct
  source 1..3683: mol_type = other DNA
ggcattgattattgactagttattaatagtaatcaattacggggtcattagttcatagcccatatatggagttccgcgttacataacttacggtaaatggcccgcctggctgaccgcccaacgacccccgcccattgacgtcaataatgacgtatgttcccatagtaacgccaatagggactttccattgacgtcaatgggtggagtatttacggtaaactgcccacttggcagtacatcaagtgtatcatatgccaagtacgccccctattgacgtcaatgacggtaaatggcccgcctggcattatgcccagtacatgaccttatgggactttcctacttggcagtacatctacgtattagtcatcgctattaccatggtcgaggtgagccccacgttctgcttcactctccccatctcccccccctccccacccccaattttgtatttatttattttttaattattttgtgcagcgatgggggcggggggggggggggggcgcgcgccaggcggggcggggcggggcgaggggcggggcggggcgaggcggagaggtgcggcggcagccaatcagagcggcgcgctccgaaagtttccttttatggcgaggcggcggcggcggcggccctataaaaagcgaagcgcgcggcgggcgggagtcgctgcgttgccttcgccccgtgccccgctccgcgccgcctcgcgccgcccgccccggctctgactgaccgcgttactcccacaggtgagcgggcgggacggcccttctcctccgggctgtaattagcgcttggtttaatgacggcttgtttcttttctgtggctgcgtgaaagccttgaggggctccgggagggccctttgtgcggggggagcggctcggggggtgcgtgcgtgtgtgtgtgcgtggggagcgccgcgtgcggctccgcgctgcccggcggctgtgagcgctgcgggcgcggcgcggggctttgtgcgctccgcagtgtgcgcgaggggagcgcggccgggggcggtgccccgcggtgcggggggctgcgaggggaacaaaggctgcgtgcggggtgtgtgcgtgggggggtgagcagggggtgtgggcgcgtcggtcgggctgcaaccccccctgcacccccctccccgagttgctgagcacggcccggcttcgggtgcggggctccgtacggggcgtggcgcggggctcgccgtgccgggcggggggtggcggcaggtgggggtgccgggcggggcggggccgcctcgggccggggagggctcgggggaggggcgcggcggcccccggagcgccggcggctgtcgaggcgcggcgagccgcagccattgccttttatggtaatcgtgcgagagggcgcagggacttcctttgtcccaaatctgtgcggagccgaaatctgggaggcgccgccgcaccccctctagcgggcgcggggcgaagcggtgcggcgccggcaggaaggaaatgggcggggagggccttcgtgcgtcgccgcgccgccgtccccttctccctctccagcctcggggctgtccgcggggggacggctgccttcgggggggacggggcagggcggggttcggcttctggcgtgtgaccggcggctctagagcctctgctaaccatgttcatgccttcttctttttcctacagctcctgggcaacgtgctggttattgtgctgtctcatcattttggcaaagaattgattaattcgagcgaacgcgtcgagtcgctcggtacgatttaaattgaattggcctcgagcgcaagcttgagctagcctcgacctcgagacgcgtgatatcggatccactagtccagtgtggtggaattcgccgccaccatgctagcccgcgcccctcctcgccgcccgccgcggctggtgctgctccgtttgctgttgctgcatctgctgctgctcgccctgcgcgcccgctgcctgagcgctgagccgggtcagggcgcgcagacctgggctcgcttcgcgcgcgctcctgccccagaggccgctggcctcctccacgacaccttccccgacggtttcctctgggcggtaggcagcgccgcctatcagaccgagggcggctggcgacagcacggcaaaggcgcgtccatctgggacactttcacccatcactctggggcggccccgtccgactccccgatcgtcgtggcgccgtcgggtgccccgtcgcctcccctgtcctccactggagatgtggccagcgatagttacaacaacgtctaccgcgacacagaggggctgcgcgaactgggggtcacccactaccgcttctccatatcgtgggcgcgggtgctccccaatggcaccgcgggcactcccaaccgcgaggggctgcgctactaccggcggctgctggagcggctgcgggagctgggcgtgcagccggtggttaccctgtaccattgggacctgccacagcgcctgcaggacacctatggcggatgggccaatcgcgccctggccgaccatttcagggattatgccgagctctgcttccgccacttcggtggtcaggtcaagtactggatcaccattgacaacccctacgtggtggcctggcacgggtatgccaccgggcgcctggccccgggcgtgaggggcagctccaggctcgggtacctggttgcccacaacctacttttggctcatgccaaagtctggcatctctacaacacctctttccgccccacacagggaggccgggtgtctatcgccttaagctcccattggatcaatcctcgaagaatgactgactataatatcagagaatgccagaagtctcttgactttgtgctaggctggtttgccaaacccatatttattgatggcgactacccagagagtatgaagaacaacctctcgtctcttctgcctgattttactgaatctgagaagaggctcatcagaggaactgctgacttttttgctctctccttcggaccaaccttgagctttcagctattggaccctaacatgaagttccgccaattggagtctcccaacctgaggcagcttctgtcttggatagatctggaatataaccaccctccaatatttattgtggaaaatggctggtttgtctcgggaaccaccaaaagggatgatgccaaatatatgtattatctcaagaagttcataatggaaaccttaaaagcaatcagactggatggggtcgacgtcattgggtacaccgcgtggtcgctcatggacggtttcgagtggcataggggctacagcatccggcgaggactcttctacgttgactttctgagtcaggacaaggagctgttgccaaagtcttcggccttgttctaccaaaagctgatagaggacaatggctttcctcctttacctgaaaaccagccccttgaagggacatttccctgtgactttgcttggggagttgttgacaactacgttcagctgagtcctttgacaaaacccagtgtcggcctcttgcttcctcactaagggccgcttccctttagtgagggttaatgcttcgagcagacatgataagatacattgatgagtttggacaaaccacaactagaatgcagtgaaaaaaatgctttatttgtgaaatttgtgatgctattgctttatttgtaaccattataagctgcaataaacaagtt

SEQ ID NO: 8 - DNA, 2494 bp, synthetic construct
  source 1..2494: mol_type = other DNA
ggcattgattattgactagttattaatagtaatcaattacggggtcattagttcatagcccatatatggagttccgcgttacataacttacggtaaatggcccgcctggctgaccgcccaacgacccccgcccattgacgtcaataatgacgtatgttcccatagtaacgccaatagggactttccattgacgtcaatgggtggagtatttacggtaaactgcccacttggcagtacatcaagtgtatcatatgccaagtccgccccctattgacgtcaatgacggtaaatggcccgcctggcattatgcccagtacatgaccttacgggactttcctacttggcagtacatctacgtattagtcatcgctattaccatggtgatgcggttttggcagtacaccaatgggcgtggatagcggtttgactcacggggatttccaagtctccaccccattgacgtcaatgggagtttgttttggcaccaaaatcaacgggactttccaaaatgtcgtaacaactgcgatcgcccgccccgttgacgcaaatgggcggtaggcgtgtacggtgggaggtctatataagcagagctctctggctaactagagaacccactgcttactggcttatcgaaattaatacgactcactatagggagacccaagctggctagaatgctcgcccgcgcccctcctcgccgcccgccgcggctggtgctgctccgtttgctgttgctgcatctgctgctgctcgccctgcgcgcccgctgcctgagcgctgagccgggtcagggcgcgcagacctgggctcgcttcgcgcgcgctcctgccccagaggccgctggcctcctccacgacaccttccccgacggtttcctctgggcggtaggcagcgccgcctatcagaccgagggcggctggcgacagcacggcaaaggcgcgtccatctgggacactttcacccatcactctggggcggccccgtccgactccccgatcgtcgtggcgccgtcgggtgccccgtcgcctcccctgtcctccactggagatgtggccagcgatagttacaacaacgtctaccgcgacacagaggggctgcgcgaactgggggtcacccactaccgcttctccatatcgtgggcgcgggtgctccccaatggcaccgcgggcactcccaaccgcgaggggctgcgctactaccggcggctgctggagcggctgcgggagctgggcgtgcagccggtggttaccctgtaccattgggacctgccacagcgcctgcaggacacctatggcggatgggccaatcgcgccctggccgaccatttcagggattatgccgagctctgcttccgccacttcggtggtcaggtcaagtactggatcaccattgacaacccctacgtggtggcctggcacgggtatgccaccgggcgcctggccccgggcgtgaggggcagctccaggctcgggtacctggttgcccacaacctacttttggctcatgccaaagtctggcatctctacaacacctctttccgccccacacagggaggccgggtgtctatcgccttaagctcccattggatcaatcctcgaagaatgactgactataatatcagagaatgccagaagtctcttgactttgtgctaggctggtttgccaaacccatatttattgatggcgactacccagagagtatgaagaacaacctctcgtctcttctgcctgattttactgaatctgagaagaggctcatcagaggaactgctgacttttttgctctctccttcggaccaaccttgagctttcagctattggaccctaacatgaagttccgccaattggagtctcccaacctgaggcagcttctgtcttggatagatctggaatataaccaccctccaatatttattgtggaaaatggctggtttgtctcgggaaccaccaaaagggatgatgccaaatatatgtattatctcaagaagttcataatggaaaccttaaaagcaatcagactggatggggtcgacgtcattgggtacaccgcgtggtcgctcatggacggtttcgagtggcataggggctacagcatccggcgaggactcttctacgttgactttctgagtcaggacaaggagctgttgccaaagtcttcggccttgttctaccaaaagctgatagaggacaatggctttcctcctttacctgaaaaccagccccttgaagggacatttccctgtgactttgcttggggagttgttgacaactacgttcagctgagtcctttgacaaaacccagtgtcggcctcttgcttcctcactaagggccgcttccctttagtgagggttaatgcttcgagcagacatgataagatacattgatgagtttggacaaaccacaactagaatgcagtgaaaaaaatgctttatttgtgaaatttgtgatgctattgctttatttgtaaccattataagctgcaataaacaagtt

SEQ ID NO: 9 - DNA, 7947 bp, synthetic construct
  source 1..7947: mol_type = other DNA
cagcagctgcgcgctcgctcgctcactgaggccgcccgggcaaagcccgggcgtcgggcgacctttggtcgcccggcctcagtgagcgagcgagcgcgcagagagggagtggccaactccatcactaggggttccttgtagttaatgattaacccgccatgctacttatctacgtagccatgctctagacatggctcgacagatctcaatattggccattagccatattattcattggttatatagcataaatcaatattggctattggccattgcatacgttgtatctatatcataatatgtacatttatattggctcatgtccaatatgaccgccatgttggcattgattattgactagttattaatagtaatcaattacggggtcattagttcatagcccatatatggagttccgcgttacataacttacggtaaatggcccgcctggctgaccgcccaacgacccccgcccattgacgtcaataatgacgtatgttcccatagtaacgccaatagggactttccattgacgtcaatgggtggagtatttacggtaaactgcccacttggcagtacatcaagtgtatcatatgccaagtacgccccctattgacgtcaatgacggtaaatggcccgcctggcattatgcccagtacatgaccttatgggactttcctacttggcagtacatctacgtattagtcatcgctattaccatggtcgaggtgagccccacgttctgcttcactctccccatctcccccccctccccacccccaattttgtatttatttattttttaattattttgtgcagcgatgggggcggggggggggggggggcgcgcgccaggcggggcggggcggggcgaggggcggggcggggcgaggcggagaggtgcggcggcagccaatcagagcggcgcgctccgaaagtttccttttatggcgaggcggcggcggcggcggccctataaaaagcgaagcgcgcggcgggcgggagtcgctgcgttgccttcgccccgtgccccgctccgcgccgcctcgcgccgcccgccccggctctgactgaccgcgttactcccacaggtgagcgggcgggacggcccttctcctccgggctgtaattagcgcttggtttaatgacggcttgtttcttttctgtggctgcgtgaaagccttgaggggctccgggagggccctttgtgcggggggagcggctcggggggtgcgtgcgtgtgtgtgtgcgtggggagcgccgcgtgcggctccgcgctgcccggcggctgtgagcgctgcgggcgcggcgcggggctttgtgcgctccgcagtgtgcgcgaggggagcgcggccgggggcggtgccccgcggtgcggggggctgcgaggggaacaaaggctgcgtgcggggtgtgtgcgtgggggggtgagcagggggtgtgggcgcgtcggtcgggctgcaaccccccctgcacccccctccccgagttgctgagcacggcccggcttcgggtgcggggctccgtacggggcgtggcgcggggctcgccgtgccgggcggggggtggcggcaggtgggggtgccgggcggggcggggccgcctcgggccggggagggctcgggggaggggcgcggcggcccccggagcgccggcggctgtcgaggcgcggcgagccgcagccattgccttttatggtaatcgtgcgagagggcgcagggacttcctttgtcccaaatctgtgcggagccgaaatctgggaggcgccgccgcaccccctctagcgggcgcggggcgaagcggtgcggcgccggcaggaaggaaatgggcggggagggccttcgtgcgtcgccgcgccgccgtccccttctccctctccagcctcggggctgtccgcggggggacggctgccttcgggggggacggggcagggcggggttcggcttctggcgtgtgaccggcggctctagagcctctgctaaccatgttcatgccttcttctttttcctacagctcctgggcaacgtgctggttattgtgctgtctcatcattttggcaaagaattgattaattcgagcgaacgcgtcgagtcgctcggtacgatttaaattgaattggcctcgagcgcaagcttgagctagcctcgacctcgagacgcgtgatatcggatccactagtccagtgtggtggaattcgccgccaccatgctagcccgcgcccctcctcgccgcccgccgcggctggtgctgctccgtttgctgttgctgcatctgctgctgctcgccctgcgcgcccgctgcctgagcgctgagccgggtcagggcgcgcagacctgggctcgcttcgcgcgcgctcctgccccagaggccgctggcctcctccacgacaccttccccgacggtttcctctgggcggtaggcagcgccgcctatcagaccgagggcggctggcgacagcacggcaaaggcgcgtccatctgggacactttcacccatcactctggggcggccccgtccgactccccgatcgtcgtggcgccgtcgggtgccccgtcgcctcccctgtcctccactggagatgtggccagcgatagttacaacaacgtctaccgcgacacagaggggctgcgcgaactgggggtcacccactaccgcttctccatatcgtgggcgcgggtgctccccaatggcaccgcgggcactcccaaccgcgaggggctgcgctactaccggcggctgctggagcggctgcgggagctgggcgtgcagccggtggttaccctgtaccattgggacctgccacagcgcctgcaggacacctatggcggatgggccaatcgcgccctggccgaccatttcagggattatgccgagctctgcttccgccacttcggtggtcaggtcaagtactggatcaccattgacaacccctacgtggtggcctggcacgggtatgccaccgggcgcctggccccgggcgtgaggggcagctccaggctcgggtacctggttgcccacaacctacttttggctcatgccaaagtctggcatctctacaacacctctttccgccccacacagggaggccgggtgtctatcgccttaagctcccattggatcaatcctcgaagaatgactgactataatatcagagaatgccagaagtctcttgactttgtgctaggctggtttgccaaacccatatttattgatggcgactacccagagagtatgaagaacaacctctcgtctcttctgcctgattttactgaatctgagaagaggctcatcagaggaactgctgacttttttgctctctccttcggaccaaccttgagctttcagctattggaccctaacatgaagttccgccaattggagtctcccaacctgaggcagcttctgtcttggatagatctggaatataaccaccctccaatatttattgtggaaaatggctggtttgtctcgggaaccaccaaaagggatgatgccaaatatatgtattatctcaagaagttcataatggaaaccttaaaagcaatcagactggatggggtcgacgtcattgggtacaccgcgtggtcgctcatggacggtttcgagtggcataggggctacagcatccggcgaggactcttctacgttgactttctgagtcaggacaaggagctgttgccaaagtcttcggccttgttctaccaaaagctgatagaggacaatggctttcctcctttacctgaaaaccagccccttgaagggacatttccctgtgactttgcttggggagttgttgacaactacgttcagctgagtcctttgacaaaacccagtgtcggcctcttgcttcctcactaagggccgcttccctttagtgagggttaatgcttcgagcagacatgataagatacattgatgagtttggacaaaccacaactagaatgcagtgaaaaaaatgctttatttgtgaaatttgtgatgctattgctttatttgtaaccattataagctgcaataaacaagttaacaacaacaattgcattcattttatgtttcaggttcagggggagatgtgggaggttttttaaagcaagtaaaacctctacaaatgtggtaaaatccgataagggactagagcatggctacgtagataagtagcatggcgggttaatcattaactacaaggaacccctagtgatggagttggccactccctctctgcgcgctcgctcgctcactgaggccgggcgaccaaaggtcgcccgacgcccgggctttgcccgggcggcctcagtgagcgagcgagcgcgccagctggcgtaatagcgaagaggcccgcaccgatcgcccttcccaacagttgcgcagcctgaatggcgaatggaattccagacgattgagcgtcaaaatgtaggtatttccatgagcgtttttccgttgcaatggctggcggtaatattgttctggatattaccagcaaggccgatagtttgagttcttctactcaggcaagtgatgttattactaatcaaagaagtattgcgacaacggttaatttgcgtgatggacagactcttttactcggtggcctcactgattataaaaacacttctcaggattctggcgtaccgttcctgtctaaaatccctttaatcggcctcctgtttagctcccgctctgattctaacgaggaaagcacgttatacgtgctcgtcaaagcaaccatagtacgcgccctgtagcggcgcattaagcgcggcgggtgtggtggttacgcgcagcgtgaccgctacacttgccagcgccctagcgcccgctcctttcgctttcttcccttcctttctcgccacgttcgccggctttccccgtcaagctctaaatcgggggctccctttagggttccgatttagtgctttacggcacctcgaccccaaaaaacttgattagggtgatggttcacgtagtgggccatcgccctgatagacggtttttcgccctttgacgttggagtccacgttctttaatagtggactcttgttccaaactggaacaacactcaaccctatctcggtctattcttttgatttataagggattttgccgatttcggcctattggttaaaaaatgagctgatttaacaaaaatttaacgcgaattttaacaaaatattaacgtctacaatttaaatatttgcttatacaatcttcctgtttttggggcttttctgattatcaaccggggtacatatgattgacatgctagttttacgattaccgttcatcgattctcttgtttgctccagactctcaggcaatgacctgatagcctttgtagagacctctcaaaaatagctaccctctccggcatgaatttatcagctagaacggttgaatatcatattgatggtgatttgactgtctccggcctttctcacccgtttgaatctttacctacacattactcaggcattgcatttaaaatatatgagggttctaaaaatttttatccttgcgttgaaataaaggcttctcccgcaaaagtattacagggtcataatgtttttggtacaaccgatttagctttatgctctgaggctttattgcttaattttgctaattctttgccttgcctgtatgatttattggatgttggaatcgcctgatgcggtattttctccttacgcatctgtgcggtatttcacaccgcatatggtgcactctcagtacaatctgctctgatgccgcatagttaagccagccccgacacccgccaacacccgctgacgcgccctgacgggcttgtctgctcccggcatccgcttacagacaagctgtgaccgtctccgggagctgcatgtgtcagaggttttcaccgtcatcaccgaaacgcgcgagacgaaagggcctcgtgatacgcctatttttataggttaatgtcatgataataatggtttcttagacgtcaggtggcacttttcggggaaatgtgcgcggaacccctatttgtttatttttctaaatacattcaaatatgtatccgctcatgagacaataaccctgataaatgcttcaataatattgaaaaaggaagagtatgagtattcaacatttccgtgtcgcccttattcccttttttgcggcattttgccttcctgtttttgctcacccagaaacgctggtgaaagtaaaagatgctgaagatcagttgggtgcacgagtgggttacatcgaactggatctcaacagcggtaagatccttgagagttttcgccccgaagaacgttttccaatgatgagcacttttaaagttctgctatgtggcgcggtattatcccgtattgacgccgggcaagagcaactcggtcgccgcatacactattctcagaatgacttggttgagtactcaccagtcacagaaaagcatcttacggatggcatgacagtaagagaattatgcagtgctgccataaccatgagtgataacactgcggccaacttacttctgacaacgatcggaggaccgaaggagctaaccgcttttttgcacaacatgggggatcatgtaactcgccttgatcgttgggaaccggagctgaatgaagccataccaaacgacgagcgtgacaccacgatgcctgtagcaatggcaacaacgttgcgcaaactattaactggcgaactacttactctagcttcccggcaacaattaatagactggatggaggcggataaagttgcaggaccacttctgcgctcggcccttccggctggctggtttattgctgataaatctggagccggtgagcgtgggtctcgcggtatcattgcagcactggggccagatggtaagccctcccgtatcgtagttatctacacgacggggagtcaggcaactatggatgaacgaaatagacagatcgctgagataggtgcctcactgattaagcattggtaactgtcagaccaagtttactcatatatactttagattgatttaaaacttcatttttaatttaaaaggatctaggtgaagatcctttttgataatctcatgaccaaaatcccttaacgtgagttttcgttccactgagcgtcagaccccgtagaaaagatcaaaggatcttcttgagatcctttttttctgcgcgtaatctgctgcttgcaaacaaaaaaaccaccgctaccagcggtggtttgtttgccggatcaagagctaccaactctttttccgaaggtaactggcttcagcagagcgcagataccaaatactgtccttctagtgtagccgtagttaggccaccacttcaagaactctgtagcaccgcctacatacctcgctctgctaatcctgttaccagtggctgctgccagtggcgataagtcgtgtcttaccgggttggactcaagacgatagttaccggataaggcgcagcggtcgggctgaacggggggttcgtgcacacagcccagcttggagcgaacgacctacaccgaactgagatacctacagcgtgagctatgagaaagcgccacgcttcccgaagggagaaaggcggacaggtatccggtaagcggcagggtcggaacaggagagcgcacgagggagcttccagggggaaacgcctggtatctttatagtcctgtcgggtttcgccacctctgacttgagcgtcgatttttgtgatgctcgtcaggggggcggagcctatggaaaaacgccagcaacgcggcctttttacggttcctggccttttgctggccttttgctcacatgttctttcctgcgttatcccctgattctgtggataaccgtattaccgcctttgagtgagctgataccgctcgccgcagccgaacgaccgagcgcagcgagtcagtgagcgaggaagcggaagagcgcccaatacgcaaaccgcctctccccgcgcgttggccgattcattaatg

SEQ ID NO: 10 - DNA, 6269 bp, synthetic construct
  source 1..6269: mol_type = other DNA
cagcagctgcgcgctcgctcgctcactgaggccgcccgggcaaagcccgggcgtcgggcgacctttggtcgcccggcctcagtgagcgagcgagcgcgcagagagggagtggccaactccatcactaggggttccttgtagttaatgattaacccgccatgctacttatctacgtagccatgctctagacatggctcgacagatctcaatattggccattagccatattattcattggttatatagcataaatcaatattggctattggccattgcatacgttgtatctatatcataatatgtacatttatattggctcatgtccaatatgaccgccatgttggcattgattattgactagttattaatagtaatcaattacggggtcattagttcatagcccatatatggagttccgcgttacataacttacggtaaatggcccgcctggctgaccgcccaacgacccccgcccattgacgtcaataatgacgtatgttcccatagtaacgccaatagggactttccattgacgtcaatgggtggagtatttacggtaaactgcccacttggcagtacatcaagtgtatcatatgccaagtacgccccctattgacgtcaatgacggtaaatggcccgcctggcattatgcccagtacatgaccttatgggactttcctacttggcagtacatctacgtattagtcatcgctattaccatggtcgaggtgagccccacgttctgcttcactctccccatctcccccccctccccacccccaattttgtatttatttattttttaattattttgtgcagcgatgggggcggggggggggggggggcgcgcgccaggcggggcggggcggggcgaggggcggggcggggcgaggcggagaggtgcggcggcagccaatcagagcggcgcgctccgaaagtttccttttatggcgaggcggcggcggcggcggccctataaaaagcgaagcgcgcggcgggcgggagtcgctgcgttgccttcgccccgtgccccgctccgcgccgcctcgcgccgcccgccccggctctgactgaccgcgttactcccacaggtgagcgggcgggacggcccttctcctccgggctgtaattagcgcttggtttaatgacggcttgtttcttttctgtggctgcgtgaaagccttgaggggctccgggagggccctttgtgcggggggagcggctcggggggtgcgtgcgtgtgtgtgtgcgtggggagcgccgcgtgcggctccgcgctgcccggcggctgtgagcgctgcgggcgcggcgcggggctttgtgcgctccgcagtgtgcgcgaggggagcgcggccgggggcggtgccccgcggtgcggggggctgcgaggggaacaaaggctgcgtgcggggtgtgtgcgtgggggggtgagcagggggtgtgggcgcgtcggtcgggctgcaaccccccctgcacccccctccccgagttgctgagcacggcccggcttcgggtgcggggctccgtacggggcgtggcgcggggctcgccgtgccgggcggggggtggcggcaggtgggggtgccgggcggggcggggccgcctcgggccggggagggctcgggggaggggcgcggcggcccccggagcgccggcggctgtcgaggcgcggcgagccgcagccattgccttttatggtaatcgtgcgagagggcgcagggacttcctttgtcccaaatctgtgcggagccgaaatctgggaggcgccgccgcaccccctctagcgggcgcggggcgaagcggtgcggcgccggcaggaaggaaatgggcggggagggccttcgtgcgtcgccgcgccgccgtccccttctccctctccagcctcggggctgtccgcggggggacggctgccttcgggggggacggggcagggcggggttcggcttctggcgtgtgaccggcggctctagagcctctgctaaccatgttcatgccttcttctttttcctacagctcctgggcaacgtgctggttattgtgctgtctcatcattttggcaaagaattgattaattcgagcgaacgcgtcgagtcgctcggtacgatttaaattgaattggcctcgagcgcaagcttgagctagcctcgacctcgagacgcgtgatatcggatccgtcgacgcggccgcttccctttagtgagggttaatgcttcgagcagacatgataagatacattgatgagtttggacaaaccacaactagaatgcagtgaaaaaaatgctttatttgtgaaatttgtgatgctattgctttatttgtaaccattataagctgcaataaacaagttaacaacaacaattgcattcattttatgtttcaggttcagggggagatgtgggaggttttttaaagcaagtaaaacctctacaaatgtggtaaaatccgataagggactagagcatggctacgtagataagtagcatggcgggttaatcattaactacaaggaacccctagtgatggagttggccactccctctctgcgcgctcgctcgctcactgaggccgggcgaccaaaggtcgcccgacgcccgggctttgcccgggcggcctcagtgagcgagcgagcgcgccagctggcgtaatagcgaagaggcccgcaccgatcgcccttcccaacagttgcgcagcctgaatggcgaatggaattccagacgattgagcgtcaaaatgtaggtatttccatgagcgtttttccgttgcaatggctggcggtaatattgttctggatattaccagcaaggccgatagtttgagttcttctactcaggcaagtgatgttattactaatcaaagaagtattgcgacaacggttaatttgcgtgatggacagactcttttactcggtggcctcactgattataaaaacacttctcaggattctggcgtaccgttcctgtctaaaatccctttaatcggcctcctgtttagctcccgctctgattctaacgaggaaagcacgttatacgtgctcgtcaaagcaaccatagtacgcgccctgtagcggcgcattaagcgcggcgggtgtggtggttacgcgcagcgtgaccgctacacttgccagcgccctagcgcccgctcctttcgctttcttcccttcctttctcgccacgttcgccggctttccccgtcaagctctaaatcgggggctccctttagggttccgatttagtgctttacggcacctcgaccccaaaaaacttgattagggtgatggttcacgtagtgggccatcgccctgatagacggtttttcgccctttgacgttggagtccacgttctttaatagtggactcttgttccaaactggaacaacactcaaccctatctcggtctattcttttgatttataagggattttgccgatttcggcctattggttaaaaaatgagctgatttaacaaaaatttaacgcgaattttaacaaaatattaacgtctacaatttaaatatttgcttatacaatcttcctgtttttggggcttttctgattatcaaccggggtacatatgattgacatgctagttttacgattaccgttcatcgattctcttgtttgctccagactctcaggcaatgacctgatagcctttgtagagacctctcaaaaatagctaccctctccggcatgaatttatcagctagaacggttgaatatcatattgatggtgatttgactgtctccggcctttctcacccgtttgaatctttacctacacattactcaggcattgcatttaaaatatatgagggttctaaaaatttttatccttgcgttgaaataaaggcttctcccgcaaaagtattacagggtcataatgtttttggtacaaccgatttagctttatgctctgaggctttattgcttaattttgctaattctttgccttgcctgtatgatttattggatgttggaatcgcctgatgcggtattttctccttacgcatctgtgcggtatttcacaccgcatatggtgcactctcagtacaatctgctctgatgccgcatagttaagccagccccgacacccgccaacacccgctgacgcgccctgacgggcttgtctgctcccggcatccgcttacagacaagctgtgaccgtctccgggagctgcatgtgtcagaggttttcaccgtcatcaccgaaacgcgcgagacgaaagggcctcgtgatacgcctatttttataggttaatgtcatgataataatggtttcttagacgtcaggtggcacttttcggggaaatgtgcgcggaacccctatttgtttatttttctaaatacattcaaatatgtatccgctcatgagacaataaccctgataaatgcttcaataatattgaaaaaggaagagtatgagtattcaacatttccgtgtcgcccttattcccttttttgcggcattttgccttcctgtttttgctcacccagaaacgctggtgaaagtaaaagatgctgaagatcagttgggtgcacgagtgggttacatcgaactggatctcaacagcggtaagatccttgagagttttcgccccgaagaacgttttccaatgatgagcacttttaaagttctgctatgtggcgcggtattatcccgtattgacgccgggcaagagcaactcggtcgccgcatacactattctcagaatgacttggttgagtactcaccagtcacagaaaagcatcttacggatggcatgacagtaagagaattatgcagtgctgccataaccatgagtgataacactgcggccaacttacttctgacaacgatcggaggaccgaaggagctaaccgcttttttgcacaacatgggggatcatgtaactcgccttgatcgttgggaaccggagctgaatgaagccataccaaacgacgagcgtgacaccacgatgcctgtagcaatggcaacaacgttgcgcaaactattaactggcgaactacttactctagcttcccggcaacaattaatagactggatggaggcggataaagttgcaggaccacttctgcgctcggcccttccggctggctggtttattgctgataaatctggagccggtgagcgtgggtctcgcggtatcattgcagcactggggccagatggtaagccctcccgtatcgtagttatctacacgacggggagtcaggcaactatggatgaacgaaatagacagatcgctgagataggtgcctcactgattaagcattggtaactgtcagaccaagtttactcatatatactttagattgatttaaaacttcatttttaatttaaaaggatctaggtgaagatcctttttgataatctcatgaccaaaatcccttaacgtgagttttcgttccactgagcgtcagaccccgtagaaaagatcaaaggatcttcttgagatcctttttttctgcgcgtaatctgctgcttgcaaacaaaaaaaccaccgctaccagcggtggtttgtttgccggatcaagagctaccaactctttttccgaaggtaactggcttcagcagagcgcagataccaaatactgtccttctagtgtagccgtagttaggccaccacttcaagaactctgtagcaccgcctacatacctcgctctgctaatcctgttaccagtggctgctgccagtggcgataagtcgtgtcttaccgggttggactcaagacgatagttaccggataaggcgcagcggtcgggctgaacggggggttcgtgcacacagcccagcttggagcgaacgacctacaccgaactgagatacctacagcgtgagctatgagaaagcgccacgcttcccgaagggagaaaggcggacaggtatccggtaagcggcagggtcggaacaggagagcgcacgagggagcttccagggggaaacgcctggtatctttatagtcctgtcgggtttcgccacctctgacttgagcgtcgatttttgtgatgctcgtcaggggggcggagcctatggaaaaacgccagcaacgcggcctttttacggttcctggccttttgctggccttttgctcacatgttctttcctgcgttatcccctgattctgtggataaccgtattaccgcctttgagtgagctgataccgctcgccgcagccgaacgaccgagcgcagcgagtcagtgagcgaggaagcggaagagcgcccaatacgcaaaccgcctctccccgcgcgttggccgattcattaatg

SEQ ID NO: 11 - DNA, 24 bp, synthetic construct
  source 1..24: mol_type = other DNA
tcataatggaaaccttaaaagcaa

SEQ ID NO: 12 - DNA, 20 bp, synthetic construct
  source 1..20: mol_type = other DNA
cactgggttttgtcaaagga

SEQ ID NO: 13 - DNA, 17 bp, synthetic construct
  source 1..17: mol_type = other DNA
caacgagcggttccgat

SEQ ID NO: 14 - DNA, 19 bp, synthetic construct
  source 1..19: mol_type = other DNA
gccacaggttccataccca